European Patent Specification EP 3 728 282 B1, published November 22, 2023. Title: 2'3' CYCLIC DINUCLEOTIDES WITH PHOSPHONATE BOND ACTIVATING THE STING ADAPTOR PROTEIN. Applicant: Birkus, Gabriel Pav, Ondrej Jandusik, Tomas Rosenberg, Ivan Nencka, Radim. The sequence listing filed with the application follows.

SEQUENCE LISTING (24 sequences)

SEQ ID NO: 1 - DNA, 75 bp, Artificial Sequence
  Synthetic construct
aaagatcttggaaagtgaaaccttggaaaacgaaactggacaaagggaaactgcagaaactgaaacaaagcttaa

SEQ ID NO: 2 - DNA, 75 bp, Artificial Sequence
  Synthetic construct
ttaagctttgtttcagtttctgcagtttccctttgtccagtttcgttttccaaggtttcactttccaagatcttt

SEQ ID NO: 3 - DNA, 20 bp, Artificial Sequence
  Synthetic construct
tgcttgctcaactctacgtc

SEQ ID NO: 4 - DNA, 20 bp, Artificial Sequence
  Synthetic construct
gtggtttgtccaaactcatc

SEQ ID NO: 5 - DNA, 31 bp, Artificial Sequence
  Synthetic construct
gtgggatccgccccagctgagatctctgcag

SEQ ID NO: 6 - DNA, 38 bp, Artificial Sequence
  Synthetic construct
tatgcggccgcctattacacagtaacctcttccttttc

SEQ ID NO: 7 - DNA, 330 bp, Artificial Sequence
  Synthetic construct
atgtcgcatcaccatcatcatcaccaccatgggatgtcggactcagaagtcaatcaagaagctaagccagaggtcaagccagaagtcaagcctgagactcacatcaatttaaaggtgtccgatggatcttcagagatcttcttcaagatcaaaaagaccactcctttaagaaggctgatggaagcgttcgctaaaagacagggtaaggaaatggactccttaagattcttgtacgacggtattagaattcaagctgatcagacccctgaagatttggacatggaggataacgatattattgaggctcaccgcgaacagattggtggatcc

SEQ ID NO: 8 - protein, 110 aa, Artificial Sequence
  Synthetic construct
MSHHHHHHHHGMSDSEVNQEAKPEVKPEVKPETHINLKVSDGSSEIFFKIKKTTPLRRLMEAFAKRQGKEMDSLRFLYDGIRIQADQTPEDLDMEDNDIIEAHREQIGGS

SEQ ID NO: 9 - protein, 204 aa, Artificial Sequence
  Synthetic construct
APAEISAVCEKGNFNVAHGLAWSYYIGYLRLILPELQARIRTYNQHYNNLLRGAVSQRLYILLPLDCGVPDNLSMADPNIRFLDKLPQQTGDRAGIKDRVYSNSIYELLENGQRAGTCVLEYATPLQTLFAMSQYSQAGFSREDRLEQAKLFCRTLEDILADAPESQNNCRLIAYQEPADDSSFSLSQEVLRHLRQEEKEEVTV

SEQ ID NO: 10 - protein, 204 aa, Artificial Sequence
  Synthetic construct
APAEISAVCEKGNFNVAHGLAWSYYIGYLRLILPELQARIRTYNQHYNNLLRGAVSQRLYILLPLDCGVPDNLSMADPNIRFLDKLPQQTADRAGIKDRVYSNSIYELLENGQRAGTCVLEYATPLQTLFAMSQYSQAGFSREDRLEQAKLFCQTLEDILADAPESQNNCRLIAYQEPADDSSFSLSQEVLRHLRQEEKEEVTV

SEQ ID NO: 11 - protein, 392 aa, Artificial Sequence
  Synthetic construct
MKYLLPTAAAGLLLLAAQPAMAMPDKLKKVLDKLRLKRKDISEAAETVNKVVERLLRRMQKRESEFKGVEQLNTGSYYEHVKISAPNEFDVMFKLEVPRIELQEYYETGAFYLVKFKRIPRGNPLSHFLEGEVLSATKMLSKFRKIIKEEVKEIKDIDVSVEKEKPGSPAVTLLIRNPEEISVDIILALESKGSWPISTKEGLPIQGWLGTKVRTNLRREPFYLVPKNAKDGNSFQGETWRLSFSHTEKYILNNHGIEKTCCESSGAKCCRKECLKLMKYLLEQLKKEFQELDAFCSYHVKTAIFHMWTQDPQDSQWDPRNLSSCFDKLLAFFLECLRTEKLDHYFIPKFNLFSQELIDRKSKEFLSKKIEYERNNGFPIFDKLLEHHHHHH

SEQ ID NO: 12 - protein, 533 aa, Homo sapiens
MQPWHGKAMQRASEAGATAPKASARNARGAPMDPNESPAAPEAALPKAGKFGPARKSGSRQKKSAPDTQERPPVRATGARAKKAPQRAQDTQPSDATSAPGAEGLEPPAAREPALSRAGSCRQRGARCSTKPRPPPGPWDVPSPGLPVSAPILVRRDAAPGASKLRAVLEKLKLSRDDISTAAGMVKGVVDHLLLRLKCDSAFRGVGLLNTGSYYEHVKISAPNEFDVMFKLEVPRIQLEEYSNTRAYYFVKFKRNPKENHLSQFLEGEILSASKMLSKFRKIVKEEINDIKDTDVIMKRKRGGSPAVTLLISEKISVDITLALESKSSWPASTQEGLRIQNWLSAKVRKQLRLKPFYLVPKHAKEGNGFQEETWRLSFSHIEKEILNNHGKSKTCCENKEEKCCRKDCLKLMKYLLEQLKERFKDKKHLDKFSSYHVKTAFFHVCTQNPQDSQWDRKDLGLCFDNCVTYFLQCLRTEKLENYFIPEFNLFSSNLIDKRSKEFLTKQIEYERNNEFPVFDEFAAALEHHHHHH

SEQ ID NO: 13 - DNA, 40 bp, Artificial sequence
  Synthetic polynucleotide
tttaagaaggagatatacatatgcagccttggcacggaaa

SEQ ID NO: 14 - DNA, 20 bp, Artificial sequence
  Synthetic polynucleotide
cttcacgtgctcatagtagc

SEQ ID NO: 15 - DNA, 40 bp, Artificial sequence
  Synthetic polynucleotide
gctactatgagcacgtgaagatttctgcacctaatgaatt

SEQ ID NO: 16 - DNA, 20 bp, Artificial sequence
  Synthetic polynucleotide
ctttaatgtcgttaatttct

SEQ ID NO: 17 - DNA, 40 bp, Artificial sequence
  Synthetic polynucleotide
agaaattaacgacattaaagatacagatgtcatcatgaag

SEQ ID NO: 18 - DNA, 20 bp, Artificial sequence
  Synthetic polynucleotide
cttggaaaccatttccttcc

SEQ ID NO: 19 - DNA, 40 bp, Artificial sequence
  Synthetic polynucleotide
ggaaggaaatggtttccaagaagaaacatggcggctatcc

SEQ ID NO: 20 - DNA, 20 bp, Artificial sequence
  Synthetic polynucleotide
ctgcaacatttctcttcttt

SEQ ID NO: 21 - DNA, 40 bp, Artificial sequence
  Synthetic polynucleotide
aaagaagagaaatgttgcaggaaagattgtttaaaactaa

SEQ ID NO: 22 - DNA, 40 bp, Artificial sequence
  Synthetic polynucleotide
tggtgctcgagtgcggccgcaaattcatcaaaaactggaa

SEQ ID NO: 23 - DNA, 20 bp, Artificial sequence
  Synthetic polynucleotide
cgatcccgcgaaattaatac

SEQ ID NO: 24 - DNA, 20 bp, Artificial sequence
  Synthetic polynucleotide
ccctcaagacccgtttagag